European Patent Application EP 4 631 520 A1, published October 15, 2025. Title: IMMUNOGENIC COMPOSITIONS OF HEPATITIS C VIRUS AND USES THEREOF. Applicant: Jaw-Ming Cherng. Application EP. The sequence listing filed with the application follows.

SEQUENCE LISTING (1 sequence)

SEQ ID NO: 1 - DNA, 1734 bp, synthetic construct
  source 1..1734: mol_type = other DNA
atgggttcctctttttctatcttccttctagcccttctctcttgcctgaccgtgcccgcgtcagcctaccaagtacgcaactcctcgggcctctaccacgtcaccaatgattgccctaactcgagtattgtgtacgagacggccgataccattctacactctccggggtgtgtcccttgcgttcgcgagggtaacaactcgaggtgttgggtggcggtggcccccacagtcgccaccagggacggcaaactccccacaacgcagcttcgacatcatatcgatctgcttgtcgggagcgccaccctttgctcggccctctatgtgggggacttgtgcgggtctgtctttcttgtcggccaactgttcaccttctcccccagacgccactggacaacgcaagactgcaactgctctatctaccccggccatataacgggtcaccgcatggcatgggatatgatgatgaactggtcccctacaacagcgctggtagtagcccagctgctcagggtcccgcaagccatcgtggatatgatcgccggtgcccactggggagtcctagcgggcatagcgtatttctccatggtagggaactgggcgaaggtcctggtagtgctgttgctgttcgccggcgtcgatgccaacaccttcaccactggggggagtgctgccaggaccacgaccggactcgtcagtcttttcagtccgggcgccaagcagaatatccagctgatgaacaccaacggcagttggcacatcaatcgcacggccttgaactgtaatgcgagcctcgacaccggctgggtggcggggctcttctaccaccacaaattcaactcctcgggctgccccgagaggatggccagctgtaaaccccttgccgattttgaccagggctggggccctatcacctacgccaacggaagcggccctgaacaccgcccctactgctggcactaccccccaaagccctgtggtgtcgtgtcagcgaagaccgtgtgtggcccagtgtattgtttcactcctagccccgtggtggtgggaacgaccaacgtgctgggcgaccctacctacggctggggtgacaatgatacggacgtcctcatccttaataacaccaggccaccgttgggcaattggttcggttgcacctggatgaactcatctggatttaccaaagtgtgcggagcgcctccttgcgtcatcggaggagtgggcaacaacaccttgcactgccccactgactgtttccgcaagcatccagaagccacatactctcggtgtggctccggtccctggatcacgcccaggtgcctggtccactatccttataggctttggcattacccttgcaccgtcaactacaccatgttcaaggtcaggatgtacgtgggaggggtcgagcacaggctggaagctgcttgcaactggacgcgaggcgagcgttgtgatctggacgacagggacaggtccgagctcagcccgctgctgctgtccaccacacagtggcaggtccttccgtgctccttcacgaccttaccagccttgaccaccggcctcatccacctccaccggaacatcgtggacgtgcaatatttgtacggggtggggtcaagcattgtgtcctgggccatcaagtgggaatacgtcatcctcttgtttctcctgcttgcagacgcgcgcatctgctcctgcttgtggatgatgttactcatatcccaagcggaggcgtaa